European Patent Application EP 4 170 039 A1, published April 26, 2023. Title: Modifying the immune response in plants. Applicant: The Sainsbury Laboratory. The sequence listing filed with the application follows.

SEQUENCE LISTING (31 sequences)

SEQ ID NO: 1 - DNA, 31 bp, Artificial Sequence
  pL0V-CDS1ns-Pikm-1_acceptor primer
ttggagtgagaccgatatcaatacgcaaacc

SEQ ID NO: 2 - DNA, 31 bp, Artificial Sequence; identical to SEQ ID NO: 1
  pL0V-CDS1ns-Pikm-1_acceptor primer

SEQ ID NO: 3 - DNA, 28 bp, Artificial Sequence
  pTL1 primer
ttggtctcaaatggaaaccggcaacaag

SEQ ID NO: 4 - DNA, 32 bp, Artificial Sequence
  pTL1 primer
ttggtctcaaagcttagaagcccggacgtttc

SEQ ID NO: 5 - DNA, 378 bp, Artificial Sequence
  Enhancer VHH - DNA sequence corresponding to the relevant VHH which was cloned into the vector.
ttgaagacataatggctcaggttcagcttgttgaatctggtggtgctcttgttcagcctggtggttctttgcgtcttagctgtgctgcttctggcttccctgtgaaccgttattctatgcgttggtaccgtcaggctccgggcaaagaacgtgaatgggttgcaggtatgagcagcgctggtgatcgtagctcttacgaggattctgtgaagggccgtttcaccatctctcgtgatgatgctcgtaacaccgtgtacctgcagatgaactctctgaagcctgaggataccgctgtgtactactgcaatgtgaacgtgggtttcgagtactggggtcagggtactcaggttaccgtttcttctggttcgttgtcttcaa

SEQ ID NO: 6 - DNA, 426 bp, Artificial Sequence
  Minimizer VHH - DNA sequence corresponding to the relevant VHH which was cloned into the vector.
ttgaagacataatggctgacgttcagcttcaagaaagcggtggtggttctgttcaagctggtggatctcttcgtcttagctgtgctgcttctggcgacaccttcagctcttattctatggcctggtttcgtcaggctcctggtaaagagtgtgagctggttagcaacatcctgcgtgatggcactactacctacgctggttcagtgaagggccgtttcaccatctcacgtgatgatgctaagaacaccgtgtacctgcagatggtcaacctgaagtctgaggataccgctcgttattactgcgctgctgattctggtactcagctgggttatgttggtgctgtgggactttcttgcctggactacgttatggattactggggtaagggtactcaggtgaccgtgtcatctggttcgttgtcttcaa

SEQ ID NO: 7 - DNA, 411 bp, Artificial Sequence
  LaG_16 VHH - DNA sequence corresponding to the relevant VHH which was cloned into the vector.
ttgaagacataatggctcaggttcagcttgttgagtctggtggtcgtcttgtgcaggctggtgattctcttcgtctttcttgtgctgctagcggccgtactttctctacttctgctatggcttggtttcgtcaggctcctggtcgtgagcgtgaattcgttgctgctattacttggaccgtgggcaacaccattcttggcgattctgttcgtggccgtttcaccatctcacgtgatcgtgctcgtaacaccgtggacctgcagatggataatcttgagcctgaggataccgccgtgtactattgctctgctcgttctcgtggttacgtgctgtctgtgcttcgttctgtggatagctatgattactggggtcagggtactcaggttaccgtttctggttcgttgtcttcaa

SEQ ID NO: 8 - DNA, 414 bp, Artificial Sequence
  LaM_4 VHH - - DNA sequence corresponding to the relevant VHH which was cloned into the vector.
ttgaagacataatggctcaggttcagcttgttgagtctggtggttctcttgttcagcctggtggaagccttcgtctttcttgtgctgcttctggccgtttcgccgagtcatcttctatgggatggtttcgtcaggctccgggcaaagagcgtgagttcgttgctgctatttcttggtcaggtggcgctaccaactacgctgattctgctaagggacgtttcaccctgtctcgtgacaataccaagaacaccgtgtacctgcagatgaacagcctgaagcctgatgataccgctgtgtattactgcgctgctaacctgggcaactacatctcttctaaccagcgtctgtacggttactggggtcagggtactcaggttaccgtttcttctcctttcactggttcgttgtcttcaa

SEQ ID NO: 9 - DNA, 32 bp, Artificial Sequence
  pJK-B2-224M primer
ttcgtctcatccttcccacacctccaaaaccg

SEQ ID NO: 10 - DNA, 35 bp, Artificial Sequence
  pJK-B2-224M primer
ttcgtctcaaggactaccattgccacagcattgta

SEQ ID NO: 11 - DNA, 406 bp, Artificial Sequence
  LaG_2 VHH - DNA sequence corresponding to the relevant VHH which was cloned into the vector.
ttggtctcaaatggctcaggttcagcttgttgaatctggtggtggtcttgttcaggctggtggttctcttagacttagctgtgctgcttctggccggaccttctctaattatgctatgggatggttcaggcaggctcctggtaaagagagagagttcgttgctgctatctcttggactggcgtgtcaacctactacgctgattctgtgaagggccgtttcaccatcagcagggataacgataagaacaccgtgtacgtgcagatgaactctctgatccctgaggacaccgctatctattactgcgctgctgttagggcccgtagcttctctgatacttactctagggtgaacgagtacgactactggggtcagggtactcaggttacagttggttcgtgagaccaa

SEQ ID NO: 12 - DNA, 376 bp, Artificial Sequence
  LaG_24 VHH - DNA sequence corresponding to the relevant VHH which was cloned into the vector.
ttggtctcaaatggctgatgtgcagcttgttgaatctggtggtggtcttgttcagcctggtggttctcttagacttagctgtgctgcttctggcgagatcgctagcattattgctatcggttggtacaggcaggctcctggtaagcagagagaatctgttgctctgatcacccggtctggcatgattacctatggtgattctgctcagggccgtttcaccatctcaagggatgatgctaagaacaccgtgtacctgcacatggatgatctggtgcctgaagataccgctgtgtactactgcaacgccaagaaggtgagcttcggagattattggggtcagggtactcaggttaccgtgtctggttcgtgagaccaa

SEQ ID NO: 13 - DNA, 217 bp, Artificial Sequence
  LaM_1 VHH - DNA sequence corresponding to the relevant VHH which was cloned into the vector.
ttggtctcaaatggctcaggttcagcttgttgaatctggtggtggtcttgtgcaggctggtgattctcttagacttagctgtgctgctagcggtaggaccttcgagaattatgctatgggatggttcaggcaggctcctggtaaagaaagggaattcgttggtgctgtgtcttggggtggtggtaggacttattacgctgacggttcgtgagaccaa

SEQ ID NO: 14 - DNA, 418 bp, Artificial Sequence
  LaM_2 VHH - DNA sequence corresponding to the relevant VHH which was cloned into the vector.
ttggtctcaaatggctcaggttcagcttgttgaatctggtggtggtcttgttcaggctggtggttctcttagacttagctgcgctactagcggcttcaccttctctgattatgctatgggatggttcaggcaggctcctggtaaagagagagagttcgttgctgccatcagctggtctggtcatgtgactgattacgccgattctgtgaagggccgtttcaccatctctagggacaatgtgaagaacaccgtgtacctgcagatgaactctctgaagcctgaggataccgctgtgtattcttgtgctgctgctaagtctggcacctggtggtatcagaggtctgagaacgatttcggttcttggggtcagggtactcaggtgaccgtttctaaagaggctattggttcgtgagaccaa

SEQ ID NO: 15 - DNA, 412 bp, Artificial Sequence
  LaM_3 VHH - DNA sequence corresponding to the relevant VHH which was cloned into the vector.
ttggtctcaaatggctcaggttcagcttgttcaatctggtggtggtcttgttcaggctggtggatctcttagacttagctgtgctgcttctggcaggaccttctctgatattgctgttggttggttcaggcagacccctggtaaagagagagagttcgttgctgccatctcttggtctggcctgatcatcaactacggcgattctgttgaggaccggttcaccatctctagggacaatgctaagtctgccgtgtacctgcagatgaactctctgaagcctgaggataccgctgtgtattattgcgctgctaggatcggcatgaactactactacgctcgtgagatcgagtacccttattggggtcagggtactcaggttaccgtgtctaagtgctacggttcgtgagaccaa

SEQ ID NO: 16 - DNA, 394 bp, Artificial Sequence
  LaM_6 VHH - DNA sequence corresponding to the relevant VHH which was cloned into the vector.
ttggtctcaaatggctcaggttcagcttgttgaatctggtggtggtcttgttcaggctggtggttctcttaggctttcttgtgtggcttctggcagcgctccttctttctttgctatggcttggtacaggcagagccctggtaatgagagagaactggttgctgctcttagcagccttggctctactaactacgctgattctgtgaagggccgtttcaccatcagcatggacaatgctaagaacaccgtgtacctgcagatgaacaacgtgaacgctgaggataccgctgtgtattattgcgctgctggcgatttccacagctgctacgctagaaagtcttgcgattattggggtcagggtactcaggttaccgtgtctggttcgtgagaccaa

SEQ ID NO: 17 - DNA, 403 bp, Artificial Sequence
  LaM_8 VHH - DNA sequence corresponding to the relevant VHH which was cloned into the vector.
ttggtctcaaatggctcaggttcagcttgttgaatctggtggtggacttgttcaggctggtggatctcttaggctttcttgcgctgtttctggcaggccattctctgagtacaaccttggatggttcaggcaggctccaggtaaagagagagagttcgttgctaggatcaggtcctctggcactactgtgtacactgattccgtgaagggccgtttctctgcttctagggataacgctaagaacatgggctacctccagctcaactctcttgagccagaggatactgctgtgtactactgcgctatgtccagggttgacacagactctccagctttctacgattactggggacagggaactcaggtgacagtttctactccaaggtccggttcgtgagaccaa

SEQ ID NO: 18 - DNA, 54 bp, Artificial Sequence
  pICH47751_mRFP1 primer
ttgaagacaacagaatcatgggtggaatgtgagaccgatatcaatacgcaaacc

SEQ ID NO: 19 - DNA, 54 bp, Artificial Sequence
  pICH47751_mRFP1 primer
ttgaagacaacatcctccttcacctgcgaatgagacctataaacgcagaaaggc

SEQ ID NO: 20 - DNA, 30 bp, Artificial Sequence
  EC15095 primer
ttgaagacaaaatggtgagcaagggcgagg

SEQ ID NO: 21 - DNA, 40 bp, Artificial Sequence
  EC15095 primer
ttgaagacaacatttgagaccacagagtgattaatgaatc

SEQ ID NO: 22 - DNA, 32 bp, Artificial Sequence; identical to SEQ ID NO: 9
  pJK-B2-099 primer

SEQ ID NO: 23 - DNA, 35 bp, Artificial Sequence; identical to SEQ ID NO: 10
  pJK-B2-099 primer

SEQ ID NO: 24 - protein, 1190 aa, Artificial Sequence
  Pikm1^Enhancer
MEAAAMAVTAATGALAPVLVKLAALLDDGECNLLEGSRSDAEFIRSELEAVHSLLTPNILGRMGDDDAACKDGLIAEVRELSYDLDDAVDDFLELNFEQRRSASPFGELKARVEERVSNRFSDWKLPAASLPPSSVHRRAGLPPPDAGLVGMHKRKEELIELLEQGSSDASRWRKRKPHVPLRIMGGMAQVQLVESGGALVQPGGSLRLSCAASGFPVNRYSMRWYRQAPGKEREWVAGMSSAGDRSSYEDSVKGRFTISRDDARNTVYLQMNSLKPEDTAVYYCNVNVGFEYWGQGTQVTVSSGSQVKEDVKEITAMLAPVKSICEFHEVKTICILGLPGGGKTTIARVLYHALGTQFQCRVFASISPSSSPSPNLTETLADIFAQAQLGVTDTLSTPYGGSGTGRALQQHLIDNISAFLLNKKYLIVIDDIWHWEEWEVIRKSIPKNDLGGRIIMTTRLNSIAEKCHTDDNDVFVYEVGDLDNNDAWSLSWGIATKSGAGNRIGTGEDNSCYDIVNMCYGMPLALIWLSSALVGEIEELGGAEVKKCRDLRHIEDGILDIPSLQPLAESLCLGYNHLPLYLRTLLLYCSAYHWSNRIERGRLVRRWIAEGFVSEEKEAEGYFGELINRGWITQHGDNNSYNYYEIHPVMLAFLRCKSKEYNFLTCLGLGSDTSTSASSPRLIRRLSLQGGYPVDCLSSMSMDVSHTCSLVVLGDVARPKGIPFYMFKRLRVLDLEDNKDIQDSHLQGICEQLSLRVRYLGLKGTRIRKLPQEMRKLKHLEILYVGSTRISELPQEIGELKHLRILDVRNTDITELPLQIRELQHLHTLDVRNTPISELPPQVGKLQNLKIMCVRSTGVRELPKEIGELNHLQTLDVRNTRVRELPWQAGQISQSLRVLAGDSGDGVRLPEGVCEALINGIPGATRAKCREVLSIAIIDRFGPPLVGIFKVPGSHMRIPKMIKDHFRVLSCLDIRLCHKLEDDDQKFLAEMPNLQTLVLRFEALPRQPITINGTGFQMLESFRVDSRVPRIAFHEDAMPNLKLLEFKFYAGPASNDAIGITNLKSLQKVVFRCSPWYKSDAPGISATIDVVKKEAEEHPNRPITLLINAGYKEISTESHGSSENIAGSSGIDTEPAQAQHDNLPAVRDDYKGKGILLDGRCPTCGRATKIEEETQDRVADIEIQTETTS

SEQ ID NO: 25 - protein, 1201 aa, Artificial Sequence
  Pikm1^LaG16
MEAAAMAVTAATGALAPVLVKLAALLDDGECNLLEGSRSDAEFIRSELEAVHSLLTPNILGRMGDDDAACKDGLIAEVRELSYDLDDAVDDFLELNFEQRRSASPFGELKARVEERVSNRFSDWKLPAASLPPSSVHRRAGLPPPDAGLVGMHKRKEELIELLEQGSSDASRWRKRKPHVPLRIMGGMAQVQLVESGGRLVQAGDSLRLSCAASGRTFSTSAMAWFRQAPGREREFVAAITWTVGNTILGDSVRGRFTISRDRARNTVDLQMDNLEPEDTAVYYCSARSRGYVLSVLRSVDSYDYWGQGTQVTVSGSQVKEDVKEITAMLAPVKSICEFHEVKTICILGLPGGGKTTIARVLYHALGTQFQCRVFASISPSSSPSPNLTETLADIFAQAQLGVTDTLSTPYGGSGTGRALQQHLIDNISAFLLNKKYLIVIDDIWHWEEWEVIRKSIPKNDLGGRIIMTTRLNSIAEKCHTDDNDVFVYEVGDLDNNDAWSLSWGIATKSGAGNRIGTGEDNSCYDIVNMCYGMPLALIWLSSALVGEIEELGGAEVKKCRDLRHIEDGILDIPSLQPLAESLCLGYNHLPLYLRTLLLYCSAYHWSNRIERGRLVRRWIAEGFVSEEKEAEGYFGELINRGWITQHGDNNSYNYYEIHPVMLAFLRCKSKEYNFLTCLGLGSDTSTSASSPRLIRRLSLQGGYPVDCLSSMSMDVSHTCSLVVLGDVARPKGIPFYMFKRLRVLDLEDNKDIQDSHLQGICEQLSLRVRYLGLKGTRIRKLPQEMRKLKHLEILYVGSTRISELPQEIGELKHLRILDVRNTDITELPLQIRELQHLHTLDVRNTPISELPPQVGKLQNLKIMCVRSTGVRELPKEIGELNHLQTLDVRNTRVRELPWQAGQISQSLRVLAGDSGDGVRLPEGVCEALINGIPGATRAKCREVLSIAIIDRFGPPLVGIFKVPGSHMRIPKMIKDHFRVLSCLDIRLCHKLEDDDQKFLAEMPNLQTLVLRFEALPRQPITINGTGFQMLESFRVDSRVPRIAFHEDAMPNLKLLEFKFYAGPASNDAIGITNLKSLQKVVFRCSPWYKSDAPGISATIDVVKKEAEEHPNRPITLLINAGYKEISTESHGSSENIAGSSGIDTEPAQAQHDNLPAVRDDYKGKGILLDGRCPTCGRATKIEEETQDRVADIEIQTETTS

SEQ ID NO: 26 - protein, 1202 aa, Artificial Sequence
  Pikm1^LaM4
MEAAAMAVTAATGALAPVLVKLAALLDDGECNLLEGSRSDAEFIRSELEAVHSLLTPNILGRMGDDDAACKDGLIAEVRELSYDLDDAVDDFLELNFEQRRSASPFGELKARVEERVSNRFSDWKLPAASLPPSSVHRRAGLPPPDAGLVGMHKRKEELIELLEQGSSDASRWRKRKPHVPLRIMGGMAQVQLVESGGSLVQPGGSLRLSCAASGRFAESSSMGWFRQAPGKEREFVAAISWSGGATNYADSAKGRFTLSRDNTKNTVYLQMNSLKPDDTAVYYCAANLGNYISSNQRLYGYWGQGTQVTVSSPFTGSQVKEDVKEITAMLAPVKSICEFHEVKTICILGLPGGGKTTIARVLYHALGTQFQCRVFASISPSSSPSPNLTETLADIFAQAQLGVTDTLSTPYGGSGTGRALQQHLIDNISAFLLNKKYLIVIDDIWHWEEWEVIRKSIPKNDLGGRIIMTTRLNSIAEKCHTDDNDVFVYEVGDLDNNDAWSLSWGIATKSGAGNRIGTGEDNSCYDIVNMCYGMPLALIWLSSALVGEIEELGGAEVKKCRDLRHIEDGILDIPSLQPLAESLCLGYNHLPLYLRTLLLYCSAYHWSNRIERGRLVRRWIAEGFVSEEKEAEGYFGELINRGWITQHGDNNSYNYYEIHPVMLAFLRCKSKEYNFLTCLGLGSDTSTSASSPRLIRRLSLQGGYPVDCLSSMSMDVSHTCSLVVLGDVARPKGIPFYMFKRLRVLDLEDNKDIQDSHLQGICEQLSLRVRYLGLKGTRIRKLPQEMRKLKHLEILYVGSTRISELPQEIGELKHLRILDVRNTDITELPLQIRELQHLHTLDVRNTPISELPPQVGKLQNLKIMCVRSTGVRELPKEIGELNHLQTLDVRNTRVRELPWQAGQISQSLRVLAGDSGDGVRLPEGVCEALINGIPGATRAKCREVLSIAIIDRFGPPLVGIFKVPGSHMRIPKMIKDHFRVLSCLDIRLCHKLEDDDQKFLAEMPNLQTLVLRFEALPRQPITINGTGFQMLESFRVDSRVPRIAFHEDAMPNLKLLEFKFYAGPASNDAIGITNLKSLQKVVFRCSPWYKSDAPGISATIDVVKKEAEEHPNRPITLLINAGYKEISTESHGSSENIAGSSGIDTEPAQAQHDNLPAVRDDYKGKGILLDGRCPTCGRATKIEEETQDRVADIEIQTETTS

SEQ ID NO: 27 - protein, 1143 aa, Artificial Sequence
  Pik-m1
MEAAAMAVTAATGALAPVLVKLAALLDDGECNLLEGSRSDAEFIRSELEAVHSLLTPNILGRMGDDDAACKDGLIAEVRELSYDLDDAVDDFLELNFEQRRSASPFGELKARVEERVSNRFSDWKLPAASLPPSSVHRRAGLPPPDAGLVGMHKRKEELIELLEQGSSDASRWRKRKPHVPLRIMGGEMQKIVFKIPMVDDKSRTKAMSLVASTVGVHSVAIAGDLRDQVVVVGDGIDSINLVSALRKKVGPAMFLEVSQVKEDVKEITAMLAPVKSICEFHEVKTICILGLPGGGKTTIARVLYHALGTQFQCRVFASISPSSSPSPNLTETLADIFAQAQLGVTDTLSTPYGGSGTGRALQQHLIDNISAFLLNKKYLIVIDDIWHWEEWEVIRKSIPKNDLGGRIIMTTRLNSIAEKCHTDDNDVFVYEVGDLDNNDAWSLSWGIATKSGAGNRIGTGEDNSCYDIVNMCYGMPLALIWLSSALVGEIEELGGAEVKKCRDLRHIEDGILDIPSLQPLAESLCLGYNHLPLYLRTLLLYCSAYHWSNRIERGRLVRRWIAEGFVSEEKEAEGYFGELINRGWITQHGDNNSYNYYEIHPVMLAFLRCKSKEYNFLTCLGLGSDTSTSASSPRLIRRLSLQGGYPVDCLSSMSMDVSHTCSLVVLGDVARPKGIPFYMFKRLRVLDLEDNKDIQDSHLQGICEQLSLRVRYLGLKGTRIRKLPQEMRKLKHLEILYVGSTRISELPQEIGELKHLRILDVRNTDITELPLQIRELQHLHTLDVRNTPISELPPQVGKLQNLKIMCVRSTGVRELPKEIGELNHLQTLDVRNTRVRELPWQAGQISQSLRVLAGDSGDGVRLPEGVCEALINGIPGATRAKCREVLSIAIIDRFGPPLVGIFKVPGSHMRIPKMIKDHFRVLSCLDIRLCHKLEDDDQKFLAEMPNLQTLVLRFEALPRQPITINGTGFQMLESFRVDSRVPRIAFHEDAMPNLKLLEFKFYAGPASNDAIGITNLKSLQKVVFRCSPWYKSDAPGISATIDVVKKEAEEHPNRPITLLINAGYKEISTESHGSSENIAGSSGIDTEPAQAQHDNLPAVRDDYKGKGILLDGRCPTCGRATKIEEETQDRVADIEIQTETTS

SEQ ID NO: 28 - protein, 183 aa, Artificial Sequence
  Pik-m1_-_CC
EAAAMAVTAATGALAPVLVKLAALLDDGECNLLEGSRSDAEFIRSELEAVHSLLTPNILGRMGDDDAACKDGLIAEVRELSYDLDDAVDDFLELNFEQRRSASPFGELKARVEERVSNRFSDWKLPAASLPPSSVHRRAGLPPPDAGLVGMHKRKEELIELLEQGSSDASRWRKRKPHVPLRI

SEQ ID NO: 29 - protein, 525 aa, Artificial Sequence
  Pik-m1_-_LRR
TCLGLGSDTSTSASSPRLIRRLSLQGGYPVDCLSSMSMDVSHTCSLVVLGDVARPKGIPFYMFKRLRVLDLEDNKDIQDSHLQGICEQLSLRVRYLGLKGTRIRKLPQEMRKLKHLEILYVGSTRISELPQEIGELKHLRILDVRNTDITELPLQIRELQHLHTLDVRNTPISELPPQVGKLQNLKIMCVRSTGVRELPKEIGELNHLQTLDVRNTRVRELPWQAGQISQSLRVLAGDSGDGVRLPEGVCEALINGIPGATRAKCREVLSIAIIDRFGPPLVGIFKVPGSHMRIPKMIKDHFRVLSCLDIRLCHKLEDDDQKFLAEMPNLQTLVLRFEALPRQPITINGTGFQMLESFRVDSRVPRIAFHEDAMPNLKLLEFKFYAGPASNDAIGITNLKSLQKVVFRCSPWYKSDAPGISATIDVVKKEAEEHPNRPITLLINAGYKEISTESHGSSENIAGSSGIDTEPAQAQHDNLPAVRDDYKGKGILLDGRCPTCGRATKIEEETQDRVADIEIQTETTS

SEQ ID NO: 30 - protein, 357 aa, Artificial Sequence
  Pik-m1_-_NB-ARC
KEDVKEITAMLAPVKSICEFHEVKTICILGLPGGGKTTIARVLYHALGTQFQCRVFASISPSSSPSPNLTETLADIFAQAQLGVTDTLSTPYGGSGTGRALQQHLIDNISAFLLNKKYLIVIDDIWHWEEWEVIRKSIPKNDLGGRIIMTTRLNSIAEKCHTDDNDVFVYEVGDLDNNDAWSLSWGIATKSGAGNRIGTGEDNSCYDIVNMCYGMPLALIWLSSALVGEIEELGGAEVKKCRDLRHIEDGILDIPSLQPLAESLCLGYNHLPLYLRTLLLYCSAYHWSNRIERGRLVRRWIAEGFVSEEKEAEGYFGELINRGWITQHGDNNSYNYYEIHPVMLAFLRCKSKEYNFL

SEQ ID NO: 31 - protein, 1021 aa, Artificial Sequence
  Pik-m2
MELVVGASEATMKSLLGKLGNLLAQEYALISGIRGDIQYINDELASMQAFLRDLSNVPEGHSHGHRMKDWMKQIRDIAYDVEDCIDDFAHRLPQDSISDAKWSFLLTKIYELWTWWPRRVIASNIAQLKVRAQQIADRRSRYGVNNPEHLDSSSSARTRAVNYEIAEYQVTSPQIIGIKEPVGMKTVMEELEVWLTNPQAENGQAVLSIVGFGGVGKTTIATALYRKVSEKFQCRASVAVSQNYDQGKVLNSILSQVSNQEQGSSTTISEKKNLTSGAKSMLKTALSLLRGNCICQPENDGNPDNTPIRLQETTDDDQNPRKLEQLLAEKSYILLIDDIWSAETWESIRSILPKNNKGGRIIVTTRFQAVGSTCSPLETDRLHTVDFLTDDESQNLFNTSICESKIRKDSNKVDEQVPEEIWKICGGLPLAIVSMAGLVACNPRKACCDWSKLCKSLFPEQETPLTLDGVTRILDCCYNDLPADLKTCLLYLSIFPKGWKISRKRLSRRWIAEGFANEKQGLTQERVAEAYFNQLTRRNLVRPMEHGSNGKVKTFQVHDMVLEYIMSKSIEENFITVVGGHWQMTAPSNKVRRLSMQSSGSNRGSSTKGLNLAQVRSLTVFGNLNHVPFHSFNYGIIQVLDLEDWKGLKERHMTEICQMLLLKYLSIRRTEISKIPSKIQKLEYLETLDIRETYVRDLPKSIVQLKRIISILGGNKNTRKGLRLPQEKSKKPIKNPSPQGKTKEPAKKGFLSQEKGKGAMKALRVLSGIEIVEESSEVAAGLHQLTGLRKLAIYKLNITKGGDTFKQLQSSIEYLGSCGLQTLAINDENSEFINSLGDMPAPPRYLVALELSGKLEKLPKWITSITTLNKLTISVTVLRTETLEILHILPSLFSLTFAFSLSAAKQDQDIIKDILENNKLDSDGEIVIPAEGFKSLKLLRFFAPLVPKLSFLDKNAMPALEIIEMRFKDFEGLFGIEILENLREVHLKVSDGAEAITKFLVNDLKVNTEKPKVFVDGIVTA